European Patent Specification EP 3 564 394 B1, published May 24, 2023. Title: Method of Preparing Libraries of Template Polynucleotides. Applicant: Gormley, Niall Anthony Smith, Geoffrey Paul Bentley, David Rigatti, Roberto. Application 11/486,953. The sequence listing filed with the application follows.

SEQUENCE LISTING (23 sequences)

SEQ ID NO: 1 - DNA, 33 bp, Artificial Sequence
  synthetic oligonucleotide
acactctttccctacacgacgctcttccgatct

SEQ ID NO: 2 - DNA, 33 bp, Artificial Sequence
  synthetic oligonucleotide
gatcggaagagctcgtatgccgtcttctgcttg

SEQ ID NO: 3 - DNA, 44 bp, Artificial Sequence
  synthetic oligonucleotide
aatgatacggcgaccaccgagatctacactctttccctacacga

SEQ ID NO: 4 - DNA, 21 bp, Artificial Sequence
  synthetic oligonucleotide
caagcagaagacggcatacga

SEQ ID NO: 5 - DNA, 296 bp, Homo sapiens
tgatacggcgaccaccgagatctacactctttccctacacgacgctcttccgatctgtggggaccgtcctgtgcattgtagggtgttcaacagcatccctgacctccacctacaagatgccagtagcgaatcccctcagccctcatctccttgccatagttgtgtcaaccaaaatcatctccacacattgttagatgtttactgggaggcagactcactcccacttgagaaccactgtactagaaatatcaccaagagaatgagatcggaagagctcgtatgccgtcttctgcttg

SEQ ID NO: 6 - DNA, 431 bp, Homo sapiens
aatgatacggcgaccaccgagatctacactctttccctacacgacgctcttccgatctgtgggctttgttctttgagaggttgcagtcaacatgattctttaagaccagaaccctgcacacttcttgggctgtatttcttacattccttttctattttaaccatatcccatcttacctacttccagcatagtggtcatatttaatttttacaaaaccattttgccacttgctgccaactatgttctttataaagcagactttgagatggaggctagtgttcagaggggatgcttaggagaactttggagattaatacttatggcaggtaagggaaggaagcaggattagacagaaatattgaactgtgatacaaagtcagcaaagactttagtcaatagatcggaagagctcgtatgccgtcttctgcttg

SEQ ID NO: 7 - DNA, 518 bp, Homo sapiens
aatgatacggcgaccaccgagatctacactctttccctacacgacgctcttccgatctttcgattcccttcaatgattattccattcgagtacattcgatgattccattcgattctatatgatgatgattgcattcgagtccgtgtattattccattccattccattagatgattccattcgagtccattcgatgattctcttcgattccgttcgataattacgcttgattccgtttgatgttgattccattcgagtccattcaatgttaattccattcgattctaagcgatgattccattcctttccattagaagatgattccattcgagaccattcgatgattgcattcaactcattcgatgacgattccattcaattctgttcaatgattccattagattccatttgatgatgagtccattcgattccatttgatgatgattccatgcgattccattagatgatgacccctttcatttccaagatcggaagagctcgtatgccgtcttctgcttg

SEQ ID NO: 8 - DNA, 387 bp, Homo sapiens
aatgatacggcgaccaccgagatctacactctttccctacacgacgctcttccgatctttaaatgctaggcatattgtgtaccccacattggtttgtagccagctctatgtcatagggcccttaccctttacctatttattgttagtataatgtccataaacaagccaatggctcagcatgaactgatgctaaagaaagctcatgcctgagtgataaattaagtgacctcagctatttctcttcagtgttgtgaaagttatttttaacagtaggtttcctggtagattctctaaccactcggtatttcacatggcccaacttggttaactcgactggttacggcaaatgctgaagatcggaagagctcgtatgccgtcttctgcttg

SEQ ID NO: 9 - DNA, 536 bp, Homo sapiens
aatgatacggcgaccaccgagatctacactctttccctacacgaagctcttccgatcttaaggaagttaggtagataatttttgtttaggccatatagctttgattttctgataacaattttataaacttagaaattttcatgtaagatacaggaatactggaagcaaaaaaaagaaggtgctttaaccttagggattgaaaaaatagtaatttaggttgaaaatgctgcttgaaagttaatgctgatagcattactacacatgatgattttttctggaaggaaagctttatctgggccttcaatttaggaatttttctctttggtttttaaaagctgccatattcacttgagcttcatgggaaagatgcaaataactaaaacaaatgaacaaaaaccatgttgaggtcaggaacttatttcaagaaagcaagttctaggttttcttttaaagtgacagtagagccttaggcctcaaaccatctacaaccatgttaacagtaagatcggaagagctcgtatgccgtcttctgcttg

SEQ ID NO: 10 - DNA, 364 bp, Homo sapiens
aatgatacggcgaccaccgagatctacactctttccctacacgacgctcttcagatcttcctgcctcagcctcccgagtagttgggattgcaggcatgtgccaccatgccctgctaatttttgtatttttaactaaaggaggggttttgccatgttggccaggctggtcttgaatgcctgacctcaggtgatccgcccacctcagcctcccagtgctgggattacaggtgtgagccactgcgcccagctgagggtaactatttttaatgtggctgatgaatgtaactatcctgtcccatgtctctgtccccagctgcagagccctcgtcgagatcggaagagctcgtatgccgtcttctgcttg

SEQ ID NO: 11 - DNA, 374 bp, Homo sapiens
aatgatacggcgaccaccgagatctacactctttccctacacgacgctcttccgatctaaggtttaaattttctatatagcctgaaaagtttgaatgtttaattcaaactaatttattgagcaatggcatttaagaaaatggaaagatacaaagggactttcatcagatgataagtggataagagagaaaaatgcagacagatgagccagagttgtgtaaaagctgggaggctagcagggccttgtagatagccaagctgactggggaacagagataaatgggagcagagatcagaaagttcatccttaccctgctgcccgtggtgaaaggagacttgcaagatcggaagagctcgtatgccgtcttctgcttg

SEQ ID NO: 12 - DNA, 379 bp, Homo sapiens
aatgatacggcgaccaccgagatctacactctttccctacacgacgctcttccgatctaaggaatctttattttctacatttgagtttggaaaactgagctagcacatctaaatccatctaattttggtcattggttttaacaagttcatcttatttttttaaacatctgatctttattttatagaatagactacacaaagtcttttggaaaattaaaatattttaacttccaacaattttcagattttacttataaaaaaatttaaaatcctctactttactcgcatctttattatttctgactttctagctacttaaagttaaggaggaaattaacctctctaagatcggaagagctcgtatgccgtcttctgcttg

SEQ ID NO: 13 - DNA, 455 bp, Homo sapiens
aatgatacggcgaccaccgagatctacactctttccctacacgacgctcttccgatctcgccataaccacagcccaggcctccgtagccacagcacccatagccatggccaccattgtagtttctgtagtagctgccacacatggtgttggttgttgaggtcatccttgggtaggaaggagtgtaggtgacttcagtatggacacttctccgcagagggccttttatatgcctcagtgaatcagaacatagcgtgcccctgcaaaaatatctctaaaggcctttcattgtgctgagaagttctggcccttacgtatctctctgatttcatatcctgctactctcctccatttatctataatgctcaaactctgctggctttttgtcttttaaaatgcagcaggtttcttctcacaataaggagatcggaagagctcgtatgccgtcttctgcttg

SEQ ID NO: 14 - DNA, 495 bp, Homo sapiens
aatgatacggcgaccaccgagatctacactctttccctacacgacgctcttccgatctagagagaagttatttaagacaagtaaggtatcaggttgtgactcaaataccacagaatctagctattgttagcaatattaagtatattttcttaaatgaaggattctccatttaccatatgccccttggataatttccagagaatttaattttttaaaaggaattttcaccaattaaattattgttttgatcaaaagaggacccactgaacaccttattcattattaaaatgtatcataaaacttaattatggagctgggtacaggggctcatgcctgtaatcccagcactttgggaggctgaggcaggaggactgcttgagtccaggagtttgagaccagcctgggtaacatggtgaaaccctgtctctacaaaaaatacaaaaaattagccaggtgtggtgagatcggaagagctcgtatgccgtcttctgcttg

SEQ ID NO: 15 - DNA, 491 bp, Homo sapiens
aatgatacggcgaccaccgagatctacactctttccctacacgacgctcttccgatctcccagggaagccaaaagattggacacccctctttcaaactataaattcctcccatagttagtttggcctatgctgggaaatgaacaagggtggctttgaggttagaagcaaaatggagtcagttaggtcagactttttttcactatcatactttttctatgtcagatttatctcacttgtaatttttgcaagggtggtttcagagccactaagcttgtggtaattttttactgcaatagaaaactaatgcattaggtaaccctctttttttccctctgattgcttgctctggggtaagccagctgccatgttgaatttttcattttgttactgagcaatcaatgggctcactgcccgacgtgcatagaggccaatactgtggcactagtttttgagaaaagatcggaagagctcgtatgccgtcttctgcttg

SEQ ID NO: 16 - DNA, 603 bp, Homo sapiens
aatgatacggcgaccaccgagatctacactctttccctacacgacgctcttccgatcttttcagattttatatgtattaactcagaacacacacctcttatcacacatattttttcatgtaatttatctaaatcttatagaaaagggtccatttgcattttctcttattagactcctgatttcaaataatatattacttatgagtatttttctgtgctgtagttattcattcttatagatatgtaacataattccttttgcaaaggtaaaaattgagctatctcttgttgaggatttgttgatctctgtctaaagtttcaaaaataaagaactttaaaagcaaaatgtaaattcctttcaagttttagtaaaattacttcaaacttagtagcttaaacaatacagatttattatgttacagttctgtaagacagaaatctgacttgatcacaccatggtaaaaccaagatactgccagggttggttttttcttggggggggtctgtgggaagagtttgtttcctttggttttccacagcccagaggctgcttgcattcctttgatcactagatcggaagagctcgtatgccgtcttctgcttg

SEQ ID NO: 17 - DNA, 442 bp, Homo sapiens
aatgatacggcgaccaccgagatctacactctttccctacacgacgctcttccgatcttattgtttagggaataatgacaaggaaaaaaagtctgtagatattcagtacagaggcacccatctttttaaatttctgaagattttttactcatgcttggttgaatccacagatgcagaacccataggttcagagggccagctgtgctttgaaaatattagcttgtgtttttattagaaagaaaactctgaggccaggcacggtggctcacgcctgtaatcccagcactttgggaggctgaggtgggcggatcacaaggtgaggagatcgagaccattctggctaacatggtgaaaccctgtctctactaaaaatacaaaaaaattagccgggcgtggtagtgagcacctagatcggaagagctcgtatgccgtcttctgcttg

SEQ ID NO: 18 - DNA, 537 bp, Homo sapiens
aatgatacggcgaccaccgagatctacactctttccctacacgacgctcttccgatctgcaattggtaaaacagtaagcaatgaaacagacacttctcaaatattccaagatggtacacgcttttcagtgtgtatgatccaataaagccattggaagtaggctttaatagtcaaaaaagactattcagttagataggaactatttgcctataactattggccaaaaataggttaaaaaattgttttaaatttgtgctttacaaaacatgtggacttttttagaaaatgtgtcaaatttcaaaagaaatatagacattatggaaaggtcagttaagcacagccctaatcctgaaaacataactatgaaagatactagctgttacttgtaaccaaaaggaaaaaaaagatattagtaaccaataattagcaaacaatgcccatatatttcctttttttttttttttttttgagacaggggcttactcaggctggatgtgatcatgagatcggaagagctcgtatgccgtcttctgcttg

SEQ ID NO: 19 - DNA, 381 bp, Homo sapiens
aatgatacggcgaccaccgagatctacactctttccctacacgacgctcttccgatctttagaagctctattatactggaaaagagatatgagacccttcctactttaagaatcaatgaagccgggtgtggtggctcacgcctgtactcccagcattttgagaggccaagctgggcagatcacctgaggtcgggagtttgagaccagcctagccaacatgatgaaatcctgtttctactaataacacaaaaattagccgggtgtggtggcgcacatctggaatcccagctactccagaggctgaggcaggaaaattgcttgaagctgggaagcagaagttgcagtgaagatcggaagagctcgtatgccgtcttctgcttg

SEQ ID NO: 20 - DNA, 650 bp, Homo sapiens
aatgatacggcgaccaccgagatctacactctttccctacacgacgctcttccgatctggctggactgaataggatagccttagctgtaaaattgggctgatctttcaaatggactcatgcttgccgaatgactcacgctcctgtttacaaatcagctctgtgaagaaatgcagagtgggaggctctgcttgccagacggagaccttagacctccaggggcggagaacggagtacttcctctggtgctcggcttcccttcctgggggcagatctctcagcttctggttggtggctctcaaaatccagacacaaggtcagctgcagccagcgtgggccctggagtagctccagttatggggcagcaatggccccctctcattttgagagctcactttgcctgtggatggttttaatccatctggataaacttgaggcccatgggaataccatatactatggtaaccatgtacactgctctaaagatgtggctgctgttgtataactttttcctttatttttgtcaatttcctattttccagagtcttgcatacccactatgtctactgtgatagtgaacgtaaaaacatacaagatgttggtgttatcctcaatctcagatcggaagagctcgtatgccgtcttctgcttg

SEQ ID NO: 21 - DNA, 605 bp, Homo sapiens
aatgatacggcgaccaccgagatctacactctttccctacacgacgctcttccgatctctgtgagaaatcaatgtctgctgtttataagccgccgggctgtgatatcctgtgagagtggccccagtggatgaagacagatgctctcaaggagcgcagatgacgcgggttccgaaggactcggcacccagcccggaggccggcaacatgggcaaggggcctctcacggctgacctgtttcctcatcagcacatcaggacaataagagctcccacttcacaggtggtgaagagccaacgtggtgaagaatgaataaagcagctcgtggaaagtgctgtgcatgaggcctggcaaccggtccctgctctgaggtcacctgccacggagctgctgacaggaccattaaaaacacaattgtgcaagtgctcacccacattcacagcagcagaatctccaccagccaagcattggagacgatccttgcatccatagacatgaacagatgagcaaaacgtggtctatacggacgatgaaatagcactcagccctaagaagaaataaaatcccgacagagagatcggaagagctcgtatgccgtcttctgctt

SEQ ID NO: 22 - DNA, 439 bp, Homo sapiens
aatgatacggcgaccaccgagatctacactctttccctacacgacgctcttccgatctgctgagaggagaggagaggctggcagggggctgatgcaggaggtgatagggctcccggtgataagaggtgagaagaacagtctctgtgtgcctagagaagagattaccagaagtctgctatctgtttgttcgcggatgtcggacaggcaggatcggtgatggcaggtcttgggggaaggattatcaggagctaaaagctgtcttcaccttggctgctaagaactcatctcggatcttcttagaattccaaatcggacttttctcctagcagtggctacatccttaacctcaaaaatacccgtattagcagatctacctccatgaaatagacaattcttgacaaactaagatcggaagagctcgtatgccgtcttctgcttg

SEQ ID NO: 23 - DNA, 698 bp, Homo sapiens
aatgatacggcgaccaccgagatctacactctttccctacacgacgctcttccgatctgttatttttcatactgatgattctagggcggttccctggacttggctgggaccagaactgtctcacagctgccagcgctccccacccccatgagaaccatcgtgctgaagatgaagagccaaagccaaactgaccagcctctgcaaccccaagcatcaccgtgtgaggacagcgtgatgtggagccgcggagaccccacgcagtgctgcgaggggcaaccacatgcaggggggcagaggtgtgggggagcaagcagatgccaccggcatgcctaggagccacagggagcatgcgggctgggcagtgatgggaatgaacgtgaactccagtcctgccccaagaagtcctccggcccctccttctcaattcagggcacaaagtggtaactgcagcatgcagaggagtcgaggagtcttccctcgtcccaggagcagcacctcgggcacagtctcggtcccacagaacagccaagtgtgggttggtggtctagagacctccgaagatccagtgggggaaggatgggcagcagagggtctactctctgaaaataaggggaagggattttccctccccactgccaaggtcccagctactggacgtgggtggagatcggaagagctcgtatgccgtcttctgcctt